European Patent Application EP 4 603 595 A1, published August 20, 2025. Title: A method for typing the immune genes and the allelic variants thereof. Applicant: ImmuneDiscover Sweden AB. The sequence listing filed with the application follows.

SEQUENCE LISTING (383 sequences)

SEQ ID NO: 1 - DNA, 52 bp, synthetic construct
  source 1..52: mol_type = other DNA
gtagcacccactgcactgacgthhhachhhgtgcctgtgctgcctgggggtg

SEQ ID NO: 2 - DNA, 52 bp, synthetic construct
  source 1..52: mol_type = other DNA
gtagcacccactgcactgacgthhhachhhgtgcctgtgctgcctggggttg

SEQ ID NO: 3 - DNA, 53 bp, synthetic construct
  source 1..53: mol_type = other DNA
gtagcacccactgcactgacgthhhachhhcctggagttggccctggatgtgg

SEQ ID NO: 4 - DNA, 55 bp, synthetic construct
  source 1..55: mol_type = other DNA
gtagcacccactgcactgacgthhhachhhgcaaaaggccctgctcaggctctgc

SEQ ID NO: 5 - DNA, 55 bp, synthetic construct
  source 1..55: mol_type = other DNA
gtagcacccactgcactgacgthhhachhhccttggccatctgtttcatggtctc

SEQ ID NO: 6 - DNA, 53 bp, synthetic construct
  source 1..53: mol_type = other DNA
gtagcacccactgcactgacgthhhachhhggcacgtaccggtcccctgcagg

SEQ ID NO: 7 - DNA, 52 bp, synthetic construct
  source 1..52: mol_type = other DNA
gtagcacccactgcactgacgthhhachhhggcagggaagggccaggtcacc

SEQ ID NO: 8 - DNA, 54 bp, synthetic construct
  source 1..54: mol_type = other DNA
gtagcacccactgcactgacgthhhachhhccctctgaagcccctgtttggagc

SEQ ID NO: 9 - DNA, 54 bp, synthetic construct
  source 1..54: mol_type = other DNA
gtagcacccactgcactgacgthhhachhhgaaggggccagggcacctgtggtc

SEQ ID NO: 10 - DNA, 53 bp, synthetic construct
  source 1..53: mol_type = other DNA
gtagcacccactgcactgacgthhhachhhctgagggaaccctccccacagag

SEQ ID NO: 11 - DNA, 50 bp, synthetic construct
  source 1..50: mol_type = other DNA
gtagcacccactgcactgacgthhhachhhcaggtcagcctcaatgggga

SEQ ID NO: 12 - DNA, 55 bp, synthetic construct
  source 1..55: mol_type = other DNA
gtagcacccactgcactgacgthhhachhhgagtgtcaggtgtggcctcagatcc

SEQ ID NO: 13 - DNA, 55 bp, synthetic construct
  source 1..55: mol_type = other DNA
gtagcacccactgcactgacgthhhachhhcccttcagcctgcccttgttcttcc

SEQ ID NO: 14 - DNA, 45 bp, synthetic construct
  source 1..45: mol_type = other DNA
cacagctcaggtatgcacgtcacgacccaggaggccccagagctc

SEQ ID NO: 15 - DNA, 50 bp, synthetic construct
  source 1..50: mol_type = other DNA
cacagctcaggtatgcacgtcacgacacagcctcagagcccctgaaggag

SEQ ID NO: 16 - DNA, 48 bp, synthetic construct
  source 1..48: mol_type = other DNA
cacagctcaggtatgcacgtcacgagctaactggggctcccagtgctc

SEQ ID NO: 17 - DNA, 53 bp, synthetic construct
  source 1..53: mol_type = other DNA
cacagctcaggtatgcacgtcacgagagacaggctcagtttcagacaacaacc

SEQ ID NO: 18 - DNA, 52 bp, synthetic construct
  source 1..52: mol_type = other DNA
cacagctcaggtatgcacgtcacgaccccctggaaatcatagtatcagcagg

SEQ ID NO: 19 - DNA, 50 bp, synthetic construct
  source 1..50: mol_type = other DNA
cacagctcaggtatgcacgtcacgaccctggaatgcacagtctcagcagg

SEQ ID NO: 20 - DNA, 48 bp, synthetic construct
  source 1..48: mol_type = other DNA
cacagctcaggtatgcacgtcacgagcgagggacagacccgagtgttc

SEQ ID NO: 21 - DNA, 48 bp, synthetic construct
  source 1..48: mol_type = other DNA
cacagctcaggtatgcacgtcacgagcgagggacagacccgagtgtcc

SEQ ID NO: 22 - DNA, 49 bp, synthetic construct
  source 1..49: mol_type = other DNA
cacagctcaggtatgcacgtcacgagggcacaggtgggcacggacactg

SEQ ID NO: 23 - DNA, 48 bp, synthetic construct
  source 1..48: mol_type = other DNA
cacagctcaggtatgcacgtcacgacctcagagccctgctgcctcctc

SEQ ID NO: 24 - DNA, 52 bp, synthetic construct
  source 1..52: mol_type = other DNA
cacagctcaggtatgcacgtcacgaccaggacagtcctcagtggcatcacag

SEQ ID NO: 25 - DNA, 49 bp, synthetic construct
  source 1..49: mol_type = other DNA
cacagctcaggtatgcacgtcacgaggtgagtcagacccacctgccctc

SEQ ID NO: 26 - DNA, 48 bp, synthetic construct
  source 1..48: mol_type = other DNA
cacagctcaggtatgcacgtcacgactgactcctgcacaccctcctgc

SEQ ID NO: 27 - DNA, 49 bp, synthetic construct
  source 1..49: mol_type = other DNA
cacagctcaggtatgcacgtcacgacactgggccacataggagctcacc

SEQ ID NO: 28 - DNA, 52 bp, synthetic construct
  source 1..52: mol_type = other DNA
cacagctcaggtatgcacgtcacgacccgatacaggcacagatgtcagctcc

SEQ ID NO: 29 - DNA, 52 bp, synthetic construct
  source 1..52: mol_type = other DNA
cacagctcaggtatgcacgtcacgacccgatacaggcacagacctcagctcc

SEQ ID NO: 30 - DNA, 50 bp, synthetic construct
  source 1..50: mol_type = other DNA
cacagctcaggtatgcacgtcacgatcagctccatccaggaccacccagc

SEQ ID NO: 31 - DNA, 48 bp, synthetic construct
  source 1..48: mol_type = other DNA
cacagctcaggtatgcacgtcacgagggaccccaatactggcacagac

SEQ ID NO: 32 - DNA, 56 bp, synthetic construct
  source 1..56: mol_type = other DNA
gtagcacccactgcactgacgthhhachhhggtgcctggacagagaagactgggag

SEQ ID NO: 33 - DNA, 52 bp, synthetic construct
  source 1..52: mol_type = other DNA
gtagcacccactgcactgacgthhhachhhggcccagcgcagaccaaggagc

SEQ ID NO: 34 - DNA, 53 bp, synthetic construct
  source 1..53: mol_type = other DNA
gtagcacccactgcactgacgthhhachhhccgggggttgttgggcattggac

SEQ ID NO: 35 - DNA, 53 bp, synthetic construct
  source 1..53: mol_type = other DNA
gtagcacccactgcactgacgthhhachhhccagagagcgggtgccttggagc

SEQ ID NO: 36 - DNA, 55 bp, synthetic construct
  source 1..55: mol_type = other DNA
gtagcacccactgcactgacgthhhachhhcctacagacaccgctcctgagacac

SEQ ID NO: 37 - DNA, 46 bp, synthetic construct
  source 1..46: mol_type = other DNA
cacagctcaggtatgcacgtcacgaccagccgcagggttttggctg

SEQ ID NO: 38 - DNA, 45 bp, synthetic construct
  source 1..45: mol_type = other DNA
cacagctcaggtatgcacgtcacgagggaccccgctgggcttcag

SEQ ID NO: 39 - DNA, 46 bp, synthetic construct
  source 1..46: mol_type = other DNA
cacagctcaggtatgcacgtcacgagacacggggctggctgccacg

SEQ ID NO: 40 - DNA, 48 bp, synthetic construct
  source 1..48: mol_type = other DNA
cacagctcaggtatgcacgtcacgaccggrctcagtctgagagggtcc

SEQ ID NO: 41 - DNA, 52 bp, synthetic construct
  source 1..52: mol_type = other DNA
cacagctcaggtatgcacgtcacgaggtctctgggtggctgggtttttgtgg

SEQ ID NO: 42 - DNA, 59 bp, synthetic construct
  source 1..59: mol_type = other DNA
gtagcacccactgcactgacgthhhachhhgctgcctcctccctggggtttctgaaacc

SEQ ID NO: 43 - DNA, 53 bp, synthetic construct
  source 1..53: mol_type = other DNA
gtagcacccactgcactgacgthhhachhhctcagccccagcacagctgcctc

SEQ ID NO: 44 - DNA, 56 bp, synthetic construct
  source 1..56: mol_type = other DNA
gtagcacccactgcactgacgthhhachhhgctgcttcccccctggggtttctgac

SEQ ID NO: 45 - DNA, 55 bp, synthetic construct
  source 1..55: mol_type = other DNA
gtagcacccactgcactgacgthhhachhhcctccatgccagcacagctgcttcc

SEQ ID NO: 46 - DNA, 56 bp, synthetic construct
  source 1..56: mol_type = other DNA
gtagcacccactgcactgacgthhhachhhgctgcctcctccttggggtttctgac

SEQ ID NO: 47 - DNA, 56 bp, synthetic construct
  source 1..56: mol_type = other DNA
gtagcacccactgcactgacgthhhachhhgctgactcctccctcagggtttctga

SEQ ID NO: 48 - DNA, 56 bp, synthetic construct
  source 1..56: mol_type = other DNA
gtagcacccactgcactgacgthhhachhhgctgcctccttcctggcgtttctgac

SEQ ID NO: 49 - DNA, 52 bp, synthetic construct
  source 1..52: mol_type = other DNA
gtagcacccactgcactgacgthhhachhhctcctcagcccggcacagctgc

SEQ ID NO: 50 - DNA, 57 bp, synthetic construct
  source 1..57: mol_type = other DNA
gtagcacccactgcactgacgthhhachhhgctgcctccttcctcagggtttctgac

SEQ ID NO: 51 - DNA, 57 bp, synthetic construct
  source 1..57: mol_type = other DNA
gtagcacccactgcactgacgthhhachhhgctgccttctcccctagggtttctgac

SEQ ID NO: 52 - DNA, 52 bp, synthetic construct
  source 1..52: mol_type = other DNA
gtagcacccactgcactgacgthhhachhhgcagaggtagggagggagcacc

SEQ ID NO: 53 - DNA, 52 bp, synthetic construct
  source 1..52: mol_type = other DNA
gtagcacccactgcactgacgthhhachhhgcagaggtggggagggagcacc

SEQ ID NO: 54 - DNA, 55 bp, synthetic construct
  source 1..55: mol_type = other DNA
gtagcacccactgcactgacgthhhachhhggacccctgcagggaggtttgtgtc

SEQ ID NO: 55 - DNA, 57 bp, synthetic construct
  source 1..57: mol_type = other DNA
gtagcacccactgcactgacgthhhachhhgcagctgatttcccccaggcattctgc

SEQ ID NO: 56 - DNA, 52 bp, synthetic construct
  source 1..52: mol_type = other DNA
gtagcacccactgcactgacgthhhachhhcccctgcagggaggtttgtgtc

SEQ ID NO: 57 - DNA, 55 bp, synthetic construct
  source 1..55: mol_type = other DNA
gtagcacccactgcactgacgthhhachhhccctcctgtcttcctgcagggacgt

SEQ ID NO: 58 - DNA, 53 bp, synthetic construct
  source 1..53: mol_type = other DNA
gtagcacccactgcactgacgthhhachhhccccatcgttcctgcagggaggt

SEQ ID NO: 59 - DNA, 57 bp, synthetic construct
  source 1..57: mol_type = other DNA
gtagcacccactgcactgacgthhhachhhcagcgttcctgcagggaggtttgtgtc

SEQ ID NO: 60 - DNA, 55 bp, synthetic construct
  source 1..55: mol_type = other DNA
gtagcacccactgcactgacgthhhachhhccctcctgtcttcctgcagcaaggt

SEQ ID NO: 61 - DNA, 55 bp, synthetic construct
  source 1..55: mol_type = other DNA
gtagcacccactgcactgacgthhhachhhccctcctgtcttcctgcagggaggt

SEQ ID NO: 62 - DNA, 52 bp, synthetic construct
  source 1..52: mol_type = other DNA
gtagcacccactgcactgacgthhhachhhgcgccccctggtggctctgtgc

SEQ ID NO: 63 - DNA, 56 bp, synthetic construct
  source 1..56: mol_type = other DNA
gtagcacccactgcactgacgthhhachhhgccgctgatttccccagcgttcctgc

SEQ ID NO: 64 - DNA, 52 bp, synthetic construct
  source 1..52: mol_type = other DNA
gtagcacccactgcactgacgthhhachhhcccagcgttcccgcagggaggt

SEQ ID NO: 65 - DNA, 53 bp, synthetic construct
  source 1..53: mol_type = other DNA
gtagcacccactgcactgacgthhhachhhctccagcgttcctgcagggaggt

SEQ ID NO: 66 - DNA, 56 bp, synthetic construct
  source 1..56: mol_type = other DNA
gtagcacccactgcactgacgthhhachhhgatgcccctgcagcgaggtttgtgtc

SEQ ID NO: 67 - DNA, 54 bp, synthetic construct
  source 1..54: mol_type = other DNA
gtagcacccactgcactgacgthhhachhhccctcctgtcttcctgcaggaggt

SEQ ID NO: 68 - DNA, 57 bp, synthetic construct
  source 1..57: mol_type = other DNA
gtagcacccactgcactgacgthhhachhhtgcagggaggtttgtgtctgggctcac

SEQ ID NO: 69 - DNA, 57 bp, synthetic construct
  source 1..57: mol_type = other DNA
gtagcacccactgcactgacgthhhachhhgcctacctgcagggaggtttttgtctg

SEQ ID NO: 70 - DNA, 57 bp, synthetic construct
  source 1..57: mol_type = other DNA
gtagcacccactgcactgacgthhhachhhtgcagggaggtttttgtctgggctcac

SEQ ID NO: 71 - DNA, 57 bp, synthetic construct
  source 1..57: mol_type = other DNA
gtagcacccactgcactgacgthhhachhhtgcacggaggtttttgtctgggctcac

SEQ ID NO: 72 - DNA, 52 bp, synthetic construct
  source 1..52: mol_type = other DNA
gtagcacccactgcactgacgthhhachhhgtggagggttttagacgggctc

SEQ ID NO: 73 - DNA, 57 bp, synthetic construct
  source 1..57: mol_type = other DNA
gtagcacccactgcactgacgthhhachhhgagcatccctgcagggaggtttgtgtc

SEQ ID NO: 74 - DNA, 53 bp, synthetic construct
  source 1..53: mol_type = other DNA
gtagcacccactgcactgacgthhhachhhgcacagctgcctcctcccacagg

SEQ ID NO: 75 - DNA, 52 bp, synthetic construct
  source 1..52: mol_type = other DNA
cacagctcaggtatgcacgtcacgagccaggccagtcatgtgagacttcacc

SEQ ID NO: 76 - DNA, 53 bp, synthetic construct
  source 1..53: mol_type = other DNA
cacagctcaggtatgcacgtcacgactcatccactcctctgtcctctccacag

SEQ ID NO: 77 - DNA, 52 bp, synthetic construct
  source 1..52: mol_type = other DNA
cacagctcaggtatgcacgtcacgactcatccacttctgtgttctctccaca

SEQ ID NO: 78 - DNA, 53 bp, synthetic construct
  source 1..53: mol_type = other DNA
cacagctcaggtatgcacgtcacgacagggagatctcatccacttctgtgttc

SEQ ID NO: 79 - DNA, 50 bp, synthetic construct
  source 1..50: mol_type = other DNA
cacagctcaggtatgcacgtcacgaccatccactcctgtgtcttctctac

SEQ ID NO: 80 - DNA, 48 bp, synthetic construct
  source 1..48: mol_type = other DNA
cacagctcaggtatgcacgtcacgacccagtgaggaggaagggatcga

SEQ ID NO: 81 - DNA, 53 bp, synthetic construct
  source 1..53: mol_type = other DNA
cacagctcaggtatgcacgtcacgagggaggggattgagtccagtcaaggtgg

SEQ ID NO: 82 - DNA, 48 bp, synthetic construct
  source 1..48: mol_type = other DNA
cacagctcaggtatgcacgtcacgactctactgtgtcctctccgcagg

SEQ ID NO: 83 - DNA, 49 bp, synthetic construct
  source 1..49: mol_type = other DNA
cacagctcaggtatgcacgtcacgactggttccagggctgaggaaggga

SEQ ID NO: 84 - DNA, 53 bp, synthetic construct
  source 1..53: mol_type = other DNA
cacagctcaggtatgcacgtcacgaccagtgatgaggaggggattgagtccag

SEQ ID NO: 85 - DNA, 53 bp, synthetic construct
  source 1..53: mol_type = other DNA
cacagctcaggtatgcacgtcacgaggaggggactgggtccagttaagtggtg

SEQ ID NO: 86 - DNA, 50 bp, synthetic construct
  source 1..50: mol_type = other DNA
cacagctcaggtatgcacgtcacgagaggattttattcacccctgtgtcc

SEQ ID NO: 87 - DNA, 48 bp, synthetic construct
  source 1..48: mol_type = other DNA
cacagctcaggtatgcacgtcacgacacccctgtgtcctctccacagg

SEQ ID NO: 88 - DNA, 50 bp, synthetic construct
  source 1..50: mol_type = other DNA
cacagctcaggtatgcacgtcacgaagctgaggaacggatcctggttcag

SEQ ID NO: 89 - DNA, 49 bp, synthetic construct
  source 1..49: mol_type = other DNA
cacagctcaggtatgcacgtcacgagctgaggaacggatcctggttcag

SEQ ID NO: 90 - DNA, 54 bp, synthetic construct
  source 1..54: mol_type = other DNA
cacagctcaggtatgcacgtcacgacagggacttcctcagaagtgaaacatcag

SEQ ID NO: 91 - DNA, 58 bp, synthetic construct
  source 1..58: mol_type = other DNA
cacagctcaggtatgcacgtcacgaggtgggcttcatcttcttatgctttctccacag

SEQ ID NO: 92 - DNA, 50 bp, synthetic construct
  source 1..50: mol_type = other DNA
cacagctcaggtatgcacgtcacgagtgctgtggtcagggactccttcac

SEQ ID NO: 93 - DNA, 58 bp, synthetic construct
  source 1..58: mol_type = other DNA
cacagctcaggtatgcacgtcacgaggtgggcttcatcttcttatgtcttctccacag

SEQ ID NO: 94 - DNA, 53 bp, synthetic construct
  source 1..53: mol_type = other DNA
cacagctcaggtatgcacgtcacgagggcttcatcttcttatgtcttctccac

SEQ ID NO: 95 - DNA, 51 bp, synthetic construct
  source 1..51: mol_type = other DNA
cacagctcaggtatgcacgtcacgagagtggacgtgagtgagataagcagt

SEQ ID NO: 96 - DNA, 51 bp, synthetic construct
  source 1..51: mol_type = other DNA
cacagctcaggtatgcacgtcacgagagagaaacagtgggtatgtgtggca

SEQ ID NO: 97 - DNA, 51 bp, synthetic construct
  source 1..51: mol_type = other DNA
cacagctcaggtatgcacgtcacgaggcagtttctgatcttagtgtctctg

SEQ ID NO: 98 - DNA, 57 bp, synthetic construct
  source 1..57: mol_type = other DNA
cacagctcaggtatgcacgtcacgacgagtgagagaaacagtggatttgtgtggcag

SEQ ID NO: 99 - DNA, 54 bp, synthetic construct
  source 1..54: mol_type = other DNA
cacagctcaggtatgcacgtcacgagcggtggatgtgtgtgacagtttctgacc

SEQ ID NO: 100 - DNA, 54 bp, synthetic construct
  source 1..54: mol_type = other DNA
cacagctcaggtatgcacgtcacgagcagtggatacgtgtggcagtttctgacc

SEQ ID NO: 101 - DNA, 56 bp, synthetic construct
  source 1..56: mol_type = other DNA
cacagctcaggtatgcacgtcacgagagagactgagtgtgagtgaacatgagtgag

SEQ ID NO: 102 - DNA, 59 bp, synthetic construct
  source 1..59: mol_type = other DNA
cacagctcaggtatgcacgtcacgagtgaacatgagtgagaaaaactggatttgtgtgg

SEQ ID NO: 103 - DNA, 54 bp, synthetic construct
  source 1..54: mol_type = other DNA
cacagctcaggtatgcacgtcacgagagatgttgagtgtgagtgaacatgagtg

SEQ ID NO: 104 - DNA, 57 bp, synthetic construct
  source 1..57: mol_type = other DNA
cacagctcaggtatgcacgtcacgagtggatatgtgtggcagtttctgaccttggtg

SEQ ID NO: 105 - DNA, 59 bp, synthetic construct
  source 1..59: mol_type = other DNA
cacagctcaggtatgcacgtcacgacagtggatatgtgtggcagtttctaaccaatgtc

SEQ ID NO: 106 - DNA, 54 bp, synthetic construct
  source 1..54: mol_type = other DNA
cacagctcaggtatgcacgtcacgagcagtggatttgtgtggcagtttctgacc

SEQ ID NO: 107 - DNA, 54 bp, synthetic construct
  source 1..54: mol_type = other DNA
cacagctcaggtatgcacgtcacgagcagtggatatgtgtggcagtttctgacc

SEQ ID NO: 108 - DNA, 57 bp, synthetic construct
  source 1..57: mol_type = other DNA
cacagctcaggtatgcacgtcacgagcagtggatttgtgtgacagtttctgaccagg

SEQ ID NO: 109 - DNA, 57 bp, synthetic construct
  source 1..57: mol_type = other DNA
cacagctcaggtatgcacgtcacgagcagtggacgtgtgtggcactttctgaccagg

SEQ ID NO: 110 - DNA, 57 bp, synthetic construct
  source 1..57: mol_type = other DNA
cacagctcaggtatgcacgtcacgagcagtggatgtgtgtggcagtttctgaccagg

SEQ ID NO: 111 - DNA, 53 bp, synthetic construct
  source 1..53: mol_type = other DNA
cacagctcaggtatgcacgtcacgagtgtggcagtttctgaccttggtgtctc

SEQ ID NO: 112 - DNA, 57 bp, synthetic construct
  source 1..57: mol_type = other DNA
cacagctcaggtatgcacgtcacgagcatgagtggatttgtgtggcagtttctgacc

SEQ ID NO: 113 - DNA, 52 bp, synthetic construct
  source 1..52: mol_type = other DNA
cacagctcaggtatgcacgtcacgagtgcctctgagcccagggctcactgtg

SEQ ID NO: 114 - DNA, 52 bp, synthetic construct
  source 1..52: mol_type = other DNA
cacagctcaggtatgcacgtcacgagtgcctctgatcccagggctcactgtg

SEQ ID NO: 115 - DNA, 49 bp, synthetic construct
  source 1..49: mol_type = other DNA
cacagctcaggtatgcacgtcacgagctgcctctgatcccagggctcac

SEQ ID NO: 116 - DNA, 52 bp, synthetic construct
  source 1..52: mol_type = other DNA
cacagctcaggtatgcacgtcacgagtgcctctgatcccagggctcaccgtg

SEQ ID NO: 117 - DNA, 52 bp, synthetic construct
  source 1..52: mol_type = other DNA
cacagctcaggtatgcacgtcacgagggctcactgtgggtctctctgttcac

SEQ ID NO: 118 - DNA, 50 bp, synthetic construct
  source 1..50: mol_type = other DNA
cacagctcaggtatgcacgtcacgaggaggtcacagaggagaacgggtgg

SEQ ID NO: 119 - DNA, 55 bp, synthetic construct
  source 1..55: mol_type = other DNA
cacagctcaggtatgcacgtcacgagcagcattcacagactgaggggtgtttcac

SEQ ID NO: 120 - DNA, 49 bp, synthetic construct
  source 1..49: mol_type = other DNA
cacagctcaggtatgcacgtcacgagcactcccatctcctctccacagg

SEQ ID NO: 121 - DNA, 48 bp, synthetic construct
  source 1..48: mol_type = other DNA
cacagctcaggtatgcacgtcacgaccactcctgtgtcccctccacag

SEQ ID NO: 122 - DNA, 56 bp, synthetic construct
  source 1..56: mol_type = other DNA
gtagcacccactgcactgacgthhhachhhgcatatcactataccactgtaccctc

SEQ ID NO: 123 - DNA, 63 bp, synthetic construct
  source 1..63: mol_type = other DNA
gtagcacccactgcactgacgthhhachhhgcagcattcactttcaaagaagtgttctgacag

SEQ ID NO: 124 - DNA, 60 bp, synthetic construct
  source 1..60: mol_type = other DNA
gtagcacccactgcactgacgthhhachhhcacatgagaactgaaatggcccaaacccag

SEQ ID NO: 125 - DNA, 63 bp, synthetic construct
  source 1..63: mol_type = other DNA
gtagcacccactgcactgacgthhhachhhctgacagatgatatgtgtaaacacatacctgtc

SEQ ID NO: 126 - DNA, 59 bp, synthetic construct
  source 1..59: mol_type = other DNA
gtagcacccactgcactgacgthhhachhhcactgtacccttcaatttacagtcatctc

SEQ ID NO: 127 - DNA, 52 bp, synthetic construct
  source 1..52: mol_type = other DNA
gtagcacccactgcactgacgthhhachhhctacaggcgcccgccactaagc

SEQ ID NO: 128 - DNA, 56 bp, synthetic construct
  source 1..56: mol_type = other DNA
gtagcacccactgcactgacgthhhachhhgctggagatcgccatggctattcctc

SEQ ID NO: 129 - DNA, 57 bp, synthetic construct
  source 1..57: mol_type = other DNA
gtagcacccactgcactgacgthhhachhhctacatcaaatccccatccaattcctc

SEQ ID NO: 130 - DNA, 60 bp, synthetic construct
  source 1..60: mol_type = other DNA
gtagcacccactgcactgacgthhhachhhggcctccatcctttagagatttgcagttgg

SEQ ID NO: 131 - DNA, 54 bp, synthetic construct
  source 1..54: mol_type = other DNA
gtagcacccactgcactgacgthhhachhhccgcttacagacagggaagggaag

SEQ ID NO: 132 - DNA, 54 bp, synthetic construct
  source 1..54: mol_type = other DNA
gtagcacccactgcactgacgthhhachhhcctaccaagtgccaggcattcagc

SEQ ID NO: 133 - DNA, 58 bp, synthetic construct
  source 1..58: mol_type = other DNA
gtagcacccactgcactgacgthhhachhhgagagttggctggtctatcttgtgtacc

SEQ ID NO: 134 - DNA, 57 bp, synthetic construct
  source 1..57: mol_type = other DNA
gtagcacccactgcactgacgthhhachhhggctctatcttgtgtaccagaagcagc

SEQ ID NO: 135 - DNA, 54 bp, synthetic construct
  source 1..54: mol_type = other DNA
gtagcacccactgcactgacgthhhachhhgtaccagaggcagccacaaggcag

SEQ ID NO: 136 - DNA, 57 bp, synthetic construct
  source 1..57: mol_type = other DNA
gtagcacccactgcactgacgthhhachhhcggctctatcttgtgtaccagaagcag

SEQ ID NO: 137 - DNA, 55 bp, synthetic construct
  source 1..55: mol_type = other DNA
gtagcacccactgcactgacgthhhachhhgcggctctatcctgtgaaccagagg

SEQ ID NO: 138 - DNA, 56 bp, synthetic construct
  source 1..56: mol_type = other DNA
gtagcacccactgcactgacgthhhachhhgtgtaccaggagtagtcacaaggcag

SEQ ID NO: 139 - DNA, 59 bp, synthetic construct
  source 1..59: mol_type = other DNA
gtagcacccactgcactgacgthhhachhhhhhachhhgggatggctcaaactgtctgc

SEQ ID NO: 140 - DNA, 53 bp, synthetic construct
  source 1..53: mol_type = other DNA
cacagctcaggtatgcacgtcacgagaccaattgtttctggaattgtgggctc

SEQ ID NO: 141 - DNA, 49 bp, synthetic construct
  source 1..49: mol_type = other DNA
cacagctcaggtatgcacgtcacgagtactaggccactccaaactgtgc

SEQ ID NO: 142 - DNA, 51 bp, synthetic construct
  source 1..51: mol_type = other DNA
cacagctcaggtatgcacgtcacgactgactcttggtggtgctggtagcag

SEQ ID NO: 143 - DNA, 49 bp, synthetic construct
  source 1..49: mol_type = other DNA
cacagctcaggtatgcacgtcacgagtactaggccactccaaaccgtgc

SEQ ID NO: 144 - DNA, 53 bp, synthetic construct
  source 1..53: mol_type = other DNA
cacagctcaggtatgcacgtcacgagaccaattatttctgggattatgggctc

SEQ ID NO: 145 - DNA, 55 bp, synthetic construct
  source 1..55: mol_type = other DNA
cacagctcaggtatgcacgtcacgacagaccaattatttctggaattgagggctc

SEQ ID NO: 146 - DNA, 51 bp, synthetic construct
  source 1..51: mol_type = other DNA
cacagctcaggtatgcacgtcacgaggtggtggtggaatatcacttcaacg

SEQ ID NO: 147 - DNA, 58 bp, synthetic construct
  source 1..58: mol_type = other DNA
cacagctcaggtatgcacgtcacgaggtagcgatgttgaactgattttgaaacatcac

SEQ ID NO: 148 - DNA, 54 bp, synthetic construct
  source 1..54: mol_type = other DNA
cacagctcaggtatgcacgtcacgagacctttgtcttgacttaacgtcagcagg

SEQ ID NO: 149 - DNA, 54 bp, synthetic construct
  source 1..54: mol_type = other DNA
cacagctcaggtatgcacgtcacgactgttggtgcttttcaagaattactgcct

SEQ ID NO: 150 - DNA, 57 bp, synthetic construct
  source 1..57: mol_type = other DNA
cacagctcaggtatgcacgtcacgactgttgatgcttttcaagaattactgccttag

SEQ ID NO: 151 - DNA, 50 bp, synthetic construct
  source 1..50: mol_type = other DNA
cacagctcaggtatgcacgtcacgaggagcgacatactaagaaatgcctc

SEQ ID NO: 152 - DNA, 54 bp, synthetic construct
  source 1..54: mol_type = other DNA
cacagctcaggtatgcacgtcacgagcaaggagtaccatactaaggaattcctc

SEQ ID NO: 153 - DNA, 50 bp, synthetic construct
  source 1..50: mol_type = other DNA
cacagctcaggtatgcacgtcacgaggggtgccatacaaaggaatacctc

SEQ ID NO: 154 - DNA, 54 bp, synthetic construct
  source 1..54: mol_type = other DNA
cacagctcaggtatgcacgtcacgagcaaggattgccatactaaggaattcctc

SEQ ID NO: 155 - DNA, 50 bp, synthetic construct; identical to SEQ ID NO: 153
  source 1..50: mol_type = other DNA

SEQ ID NO: 156 - DNA, 54 bp, synthetic construct
  source 1..54: mol_type = other DNA
cacagctcaggtatgcacgtcacgagcaagggataccatactaagaaatgcctc

SEQ ID NO: 157 - DNA, 48 bp, synthetic construct
  source 1..48: mol_type = other DNA
cacagctcaggtatgcacgtcacgagctcccccaatcactttggactg

SEQ ID NO: 158 - DNA, 59 bp, synthetic construct
  source 1..59: mol_type = other DNA
ggagttcagacgtgtgctcttccgatctgagacatttgtagcacccactgcactgacgt

SEQ ID NO: 159 - DNA, 59 bp, synthetic construct
  source 1..59: mol_type = other DNA
ggagttcagacgtgtgctcttccgatctgccacatttgtagcacccactgcactgacgt

SEQ ID NO: 160 - DNA, 59 bp, synthetic construct
  source 1..59: mol_type = other DNA
ggagttcagacgtgtgctcttccgatctgctacagttgtagcacccactgcactgacgt

SEQ ID NO: 161 - DNA, 59 bp, synthetic construct
  source 1..59: mol_type = other DNA
ggagttcagacgtgtgctcttccgatctggcacacttgtagcacccactgcactgacgt

SEQ ID NO: 162 - DNA, 59 bp, synthetic construct
  source 1..59: mol_type = other DNA
ggagttcagacgtgtgctcttccgatctcggacaattgtagcacccactgcactgacgt

SEQ ID NO: 163 - DNA, 59 bp, synthetic construct
  source 1..59: mol_type = other DNA
ggagttcagacgtgtgctcttccgatctactacatgtgtagcacccactgcactgacgt

SEQ ID NO: 164 - DNA, 59 bp, synthetic construct
  source 1..59: mol_type = other DNA
ggagttcagacgtgtgctcttccgatctagtacaagtgtagcacccactgcactgacgt

SEQ ID NO: 165 - DNA, 59 bp, synthetic construct
  source 1..59: mol_type = other DNA
ggagttcagacgtgtgctcttccgatctaccacaagtgtagcacccactgcactgacgt

SEQ ID NO: 166 - DNA, 59 bp, synthetic construct
  source 1..59: mol_type = other DNA
ggagttcagacgtgtgctcttccgatctacgacagctgtagcacccactgcactgacgt

SEQ ID NO: 167 - DNA, 59 bp, synthetic construct
  source 1..59: mol_type = other DNA
ggagttcagacgtgtgctcttccgatctctcacagctgtagcacccactgcactgacgt

SEQ ID NO: 168 - DNA, 59 bp, synthetic construct
  source 1..59: mol_type = other DNA
ggagttcagacgtgtgctcttccgatctacaacagctgtagcacccactgcactgacgt

SEQ ID NO: 169 - DNA, 59 bp, synthetic construct
  source 1..59: mol_type = other DNA
ggagttcagacgtgtgctcttccgatctgaaacagctgtagcacccactgcactgacgt

SEQ ID NO: 170 - DNA, 59 bp, synthetic construct
  source 1..59: mol_type = other DNA
ggagttcagacgtgtgctcttccgatctatcacacctgtagcacccactgcactgacgt

SEQ ID NO: 171 - DNA, 59 bp, synthetic construct
  source 1..59: mol_type = other DNA
ggagttcagacgtgtgctcttccgatctgacacacctgtagcacccactgcactgacgt

SEQ ID NO: 172 - DNA, 59 bp, synthetic construct
  source 1..59: mol_type = other DNA
ggagttcagacgtgtgctcttccgatctcttacaactgtagcacccactgcactgacgt

SEQ ID NO: 173 - DNA, 59 bp, synthetic construct
  source 1..59: mol_type = other DNA
ggagttcagacgtgtgctcttccgatcttgtacaactgtagcacccactgcactgacgt

SEQ ID NO: 174 - DNA, 59 bp, synthetic construct
  source 1..59: mol_type = other DNA
ggagttcagacgtgtgctcttccgatctagtacaactgtagcacccactgcactgacgt

SEQ ID NO: 175 - DNA, 59 bp, synthetic construct
  source 1..59: mol_type = other DNA
ggagttcagacgtgtgctcttccgatctgacacatatgtagcacccactgcactgacgt

SEQ ID NO: 176 - DNA, 59 bp, synthetic construct
  source 1..59: mol_type = other DNA
ggagttcagacgtgtgctcttccgatcttaaacatatgtagcacccactgcactgacgt

SEQ ID NO: 177 - DNA, 59 bp, synthetic construct
  source 1..59: mol_type = other DNA
ggagttcagacgtgtgctcttccgatctttcacagatgtagcacccactgcactgacgt

SEQ ID NO: 178 - DNA, 59 bp, synthetic construct
  source 1..59: mol_type = other DNA
ggagttcagacgtgtgctcttccgatctgacacacatgtagcacccactgcactgacgt

SEQ ID NO: 179 - DNA, 59 bp, synthetic construct
  source 1..59: mol_type = other DNA
ggagttcagacgtgtgctcttccgatctctaacacatgtagcacccactgcactgacgt

SEQ ID NO: 180 - DNA, 59 bp, synthetic construct
  source 1..59: mol_type = other DNA
ggagttcagacgtgtgctcttccgatctataacacatgtagcacccactgcactgacgt

SEQ ID NO: 181 - DNA, 59 bp, synthetic construct
  source 1..59: mol_type = other DNA
ggagttcagacgtgtgctcttccgatctcgaacacatgtagcacccactgcactgacgt

SEQ ID NO: 182 - DNA, 59 bp, synthetic construct
  source 1..59: mol_type = other DNA
ggagttcagacgtgtgctcttccgatcttgtacaaatgtagcacccactgcactgacgt

SEQ ID NO: 183 - DNA, 59 bp, synthetic construct
  source 1..59: mol_type = other DNA
ggagttcagacgtgtgctcttccgatctgctacaaatgtagcacccactgcactgacgt

SEQ ID NO: 184 - DNA, 59 bp, synthetic construct
  source 1..59: mol_type = other DNA
ggagttcagacgtgtgctcttccgatctcggacaaatgtagcacccactgcactgacgt

SEQ ID NO: 185 - DNA, 59 bp, synthetic construct
  source 1..59: mol_type = other DNA
ggagttcagacgtgtgctcttccgatctactacattggtagcacccactgcactgacgt

SEQ ID NO: 186 - DNA, 59 bp, synthetic construct
  source 1..59: mol_type = other DNA
ggagttcagacgtgtgctcttccgatctgcaacattggtagcacccactgcactgacgt

SEQ ID NO: 187 - DNA, 59 bp, synthetic construct
  source 1..59: mol_type = other DNA
ggagttcagacgtgtgctcttccgatctccgacagtggtagcacccactgcactgacgt

SEQ ID NO: 188 - DNA, 59 bp, synthetic construct
  source 1..59: mol_type = other DNA
ggagttcagacgtgtgctcttccgatctaaaacagtggtagcacccactgcactgacgt

SEQ ID NO: 189 - DNA, 59 bp, synthetic construct
  source 1..59: mol_type = other DNA
ggagttcagacgtgtgctcttccgatctcgcacactggtagcacccactgcactgacgt

SEQ ID NO: 190 - DNA, 59 bp, synthetic construct
  source 1..59: mol_type = other DNA
ggagttcagacgtgtgctcttccgatctctgacaatggtagcacccactgcactgacgt

SEQ ID NO: 191 - DNA, 59 bp, synthetic construct
  source 1..59: mol_type = other DNA
ggagttcagacgtgtgctcttccgatctgagacaatggtagcacccactgcactgacgt

SEQ ID NO: 192 - DNA, 59 bp, synthetic construct
  source 1..59: mol_type = other DNA
ggagttcagacgtgtgctcttccgatctcgaacatgggtagcacccactgcactgacgt

SEQ ID NO: 193 - DNA, 59 bp, synthetic construct
  source 1..59: mol_type = other DNA
ggagttcagacgtgtgctcttccgatctcatacacgggtagcacccactgcactgacgt

SEQ ID NO: 194 - DNA, 59 bp, synthetic construct
  source 1..59: mol_type = other DNA
ggagttcagacgtgtgctcttccgatctcacacaagggtagcacccactgcactgacgt

SEQ ID NO: 195 - DNA, 59 bp, synthetic construct
  source 1..59: mol_type = other DNA
ggagttcagacgtgtgctcttccgatctatcacagcggtagcacccactgcactgacgt

SEQ ID NO: 196 - DNA, 59 bp, synthetic construct
  source 1..59: mol_type = other DNA
ggagttcagacgtgtgctcttccgatcttaaacaccggtagcacccactgcactgacgt

SEQ ID NO: 197 - DNA, 59 bp, synthetic construct
  source 1..59: mol_type = other DNA
ggagttcagacgtgtgctcttccgatcttagacataggtagcacccactgcactgacgt

SEQ ID NO: 198 - DNA, 59 bp, synthetic construct
  source 1..59: mol_type = other DNA
ggagttcagacgtgtgctcttccgatctgacacataggtagcacccactgcactgacgt

SEQ ID NO: 199 - DNA, 59 bp, synthetic construct
  source 1..59: mol_type = other DNA
ggagttcagacgtgtgctcttccgatctggtacagaggtagcacccactgcactgacgt

SEQ ID NO: 200 - DNA, 59 bp, synthetic construct
  source 1..59: mol_type = other DNA
ggagttcagacgtgtgctcttccgatctatcacagaggtagcacccactgcactgacgt

SEQ ID NO: 201 - DNA, 59 bp, synthetic construct
  source 1..59: mol_type = other DNA
ggagttcagacgtgtgctcttccgatcttcaacagaggtagcacccactgcactgacgt

SEQ ID NO: 202 - DNA, 59 bp, synthetic construct
  source 1..59: mol_type = other DNA
ggagttcagacgtgtgctcttccgatctagtacacaggtagcacccactgcactgacgt

SEQ ID NO: 203 - DNA, 59 bp, synthetic construct
  source 1..59: mol_type = other DNA
ggagttcagacgtgtgctcttccgatctgctacaaaggtagcacccactgcactgacgt

SEQ ID NO: 204 - DNA, 59 bp, synthetic construct
  source 1..59: mol_type = other DNA
ggagttcagacgtgtgctcttccgatcttcgacaaaggtagcacccactgcactgacgt

SEQ ID NO: 205 - DNA, 59 bp, synthetic construct
  source 1..59: mol_type = other DNA
ggagttcagacgtgtgctcttccgatctatgacattcgtagcacccactgcactgacgt

SEQ ID NO: 206 - DNA, 59 bp, synthetic construct
  source 1..59: mol_type = other DNA
ggagttcagacgtgtgctcttccgatctccaacattcgtagcacccactgcactgacgt

SEQ ID NO: 207 - DNA, 59 bp, synthetic construct
  source 1..59: mol_type = other DNA
ggagttcagacgtgtgctcttccgatctagaacactcgtagcacccactgcactgacgt

SEQ ID NO: 208 - DNA, 59 bp, synthetic construct
  source 1..59: mol_type = other DNA
ggagttcagacgtgtgctcttccgatctcatacaatcgtagcacccactgcactgacgt

SEQ ID NO: 209 - DNA, 59 bp, synthetic construct
  source 1..59: mol_type = other DNA
ggagttcagacgtgtgctcttccgatcttcgacaatcgtagcacccactgcactgacgt

SEQ ID NO: 210 - DNA, 59 bp, synthetic construct
  source 1..59: mol_type = other DNA
ggagttcagacgtgtgctcttccgatctgccacaatcgtagcacccactgcactgacgt

SEQ ID NO: 211 - DNA, 59 bp, synthetic construct
  source 1..59: mol_type = other DNA
ggagttcagacgtgtgctcttccgatctgatacatgcgtagcacccactgcactgacgt

SEQ ID NO: 212 - DNA, 59 bp, synthetic construct
  source 1..59: mol_type = other DNA
ggagttcagacgtgtgctcttccgatctatcacatgcgtagcacccactgcactgacgt

SEQ ID NO: 213 - DNA, 59 bp, synthetic construct
  source 1..59: mol_type = other DNA
ggagttcagacgtgtgctcttccgatctgcaacatgcgtagcacccactgcactgacgt

SEQ ID NO: 214 - DNA, 59 bp, synthetic construct
  source 1..59: mol_type = other DNA
ggagttcagacgtgtgctcttccgatcttttacaggcgtagcacccactgcactgacgt

SEQ ID NO: 215 - DNA, 59 bp, synthetic construct
  source 1..59: mol_type = other DNA
ggagttcagacgtgtgctcttccgatcttaaacaggcgtagcacccactgcactgacgt

SEQ ID NO: 216 - DNA, 59 bp, synthetic construct
  source 1..59: mol_type = other DNA
ggagttcagacgtgtgctcttccgatctgcaacacgcgtagcacccactgcactgacgt

SEQ ID NO: 217 - DNA, 59 bp, synthetic construct
  source 1..59: mol_type = other DNA
ggagttcagacgtgtgctcttccgatcttgtacaagcgtagcacccactgcactgacgt

SEQ ID NO: 218 - DNA, 59 bp, synthetic construct
  source 1..59: mol_type = other DNA
ggagttcagacgtgtgctcttccgatctggtacatccgtagcacccactgcactgacgt

SEQ ID NO: 219 - DNA, 59 bp, synthetic construct
  source 1..59: mol_type = other DNA
ggagttcagacgtgtgctcttccgatctaatacatccgtagcacccactgcactgacgt

SEQ ID NO: 220 - DNA, 59 bp, synthetic construct
  source 1..59: mol_type = other DNA
ggagttcagacgtgtgctcttccgatctcctacagccgtagcacccactgcactgacgt

SEQ ID NO: 221 - DNA, 59 bp, synthetic construct
  source 1..59: mol_type = other DNA
ggagttcagacgtgtgctcttccgatctaaaacagccgtagcacccactgcactgacgt

SEQ ID NO: 222 - DNA, 59 bp, synthetic construct
  source 1..59: mol_type = other DNA
ggagttcagacgtgtgctcttccgatctacaacaaccgtagcacccactgcactgacgt

SEQ ID NO: 223 - DNA, 59 bp, synthetic construct
  source 1..59: mol_type = other DNA
ggagttcagacgtgtgctcttccgatcttttacatacgtagcacccactgcactgacgt

SEQ ID NO: 224 - DNA, 59 bp, synthetic construct
  source 1..59: mol_type = other DNA
ggagttcagacgtgtgctcttccgatctcggacatacgtagcacccactgcactgacgt

SEQ ID NO: 225 - DNA, 59 bp, synthetic construct
  source 1..59: mol_type = other DNA
ggagttcagacgtgtgctcttccgatctagcacatacgtagcacccactgcactgacgt

SEQ ID NO: 226 - DNA, 59 bp, synthetic construct
  source 1..59: mol_type = other DNA
ggagttcagacgtgtgctcttccgatctactacagacgtagcacccactgcactgacgt

SEQ ID NO: 227 - DNA, 59 bp, synthetic construct
  source 1..59: mol_type = other DNA
ggagttcagacgtgtgctcttccgatctgcgacagacgtagcacccactgcactgacgt

SEQ ID NO: 228 - DNA, 59 bp, synthetic construct
  source 1..59: mol_type = other DNA
ggagttcagacgtgtgctcttccgatctctaacagacgtagcacccactgcactgacgt

SEQ ID NO: 229 - DNA, 59 bp, synthetic construct
  source 1..59: mol_type = other DNA
ggagttcagacgtgtgctcttccgatctactacacacgtagcacccactgcactgacgt

SEQ ID NO: 230 - DNA, 59 bp, synthetic construct
  source 1..59: mol_type = other DNA
ggagttcagacgtgtgctcttccgatcttagacacacgtagcacccactgcactgacgt

SEQ ID NO: 231 - DNA, 59 bp, synthetic construct
  source 1..59: mol_type = other DNA
ggagttcagacgtgtgctcttccgatctggcacacacgtagcacccactgcactgacgt

SEQ ID NO: 232 - DNA, 59 bp, synthetic construct
  source 1..59: mol_type = other DNA
ggagttcagacgtgtgctcttccgatcttgaacacacgtagcacccactgcactgacgt

SEQ ID NO: 233 - DNA, 59 bp, synthetic construct
  source 1..59: mol_type = other DNA
ggagttcagacgtgtgctcttccgatctgaatctaacgtagcacccactgcactgacgt

SEQ ID NO: 234 - DNA, 59 bp, synthetic construct
  source 1..59: mol_type = other DNA
ggagttcagacgtgtgctcttccgatctatcacaaacgtagcacccactgcactgacgt

SEQ ID NO: 235 - DNA, 59 bp, synthetic construct
  source 1..59: mol_type = other DNA
ggagttcagacgtgtgctcttccgatcttccacattagtagcacccactgcactgacgt

SEQ ID NO: 236 - DNA, 59 bp, synthetic construct
  source 1..59: mol_type = other DNA
ggagttcagacgtgtgctcttccgatctactacagtagtagcacccactgcactgacgt

SEQ ID NO: 237 - DNA, 59 bp, synthetic construct
  source 1..59: mol_type = other DNA
ggagttcagacgtgtgctcttccgatctcgaacagtagtagcacccactgcactgacgt

SEQ ID NO: 238 - DNA, 59 bp, synthetic construct
  source 1..59: mol_type = other DNA
ggagttcagacgtgtgctcttccgatctgcaacactagtagcacccactgcactgacgt

SEQ ID NO: 239 - DNA, 59 bp, synthetic construct
  source 1..59: mol_type = other DNA
ggagttcagacgtgtgctcttccgatcttgcacaatagtagcacccactgcactgacgt

SEQ ID NO: 240 - DNA, 59 bp, synthetic construct
  source 1..59: mol_type = other DNA
ggagttcagacgtgtgctcttccgatctcctacatgagtagcacccactgcactgacgt

SEQ ID NO: 241 - DNA, 59 bp, synthetic construct
  source 1..59: mol_type = other DNA
ggagttcagacgtgtgctcttccgatcttgcacatgagtagcacccactgcactgacgt

SEQ ID NO: 242 - DNA, 59 bp, synthetic construct
  source 1..59: mol_type = other DNA
ggagttcagacgtgtgctcttccgatctaacacatgagtagcacccactgcactgacgt

SEQ ID NO: 243 - DNA, 59 bp, synthetic construct
  source 1..59: mol_type = other DNA
ggagttcagacgtgtgctcttccgatctagtacatcagtagcacccactgcactgacgt

SEQ ID NO: 244 - DNA, 59 bp, synthetic construct
  source 1..59: mol_type = other DNA
ggagttcagacgtgtgctcttccgatcttagacatcagtagcacccactgcactgacgt

SEQ ID NO: 245 - DNA, 59 bp, synthetic construct
  source 1..59: mol_type = other DNA
ggagttcagacgtgtgctcttccgatctcgcacatcagtagcacccactgcactgacgt

SEQ ID NO: 246 - DNA, 59 bp, synthetic construct
  source 1..59: mol_type = other DNA
ggagttcagacgtgtgctcttccgatcttatacagcagtagcacccactgcactgacgt

SEQ ID NO: 247 - DNA, 59 bp, synthetic construct
  source 1..59: mol_type = other DNA
ggagttcagacgtgtgctcttccgatctgaaacagcagtagcacccactgcactgacgt

SEQ ID NO: 248 - DNA, 59 bp, synthetic construct
  source 1..59: mol_type = other DNA
ggagttcagacgtgtgctcttccgatctcttacaccagtagcacccactgcactgacgt

SEQ ID NO: 249 - DNA, 59 bp, synthetic construct
  source 1..59: mol_type = other DNA
ggagttcagacgtgtgctcttccgatctacaacaccagtagcacccactgcactgacgt

SEQ ID NO: 250 - DNA, 59 bp, synthetic construct
  source 1..59: mol_type = other DNA
ggagttcagacgtgtgctcttccgatctgtgacaacagtagcacccactgcactgacgt

SEQ ID NO: 251 - DNA, 59 bp, synthetic construct
  source 1..59: mol_type = other DNA
ggagttcagacgtgtgctcttccgatctgggacaacagtagcacccactgcactgacgt

SEQ ID NO: 252 - DNA, 59 bp, synthetic construct
  source 1..59: mol_type = other DNA
ggagttcagacgtgtgctcttccgatcttagacaacagtagcacccactgcactgacgt

SEQ ID NO: 253 - DNA, 59 bp, synthetic construct
  source 1..59: mol_type = other DNA
ggagttcagacgtgtgctcttccgatctaacacaacagtagcacccactgcactgacgt

SEQ ID NO: 254 - DNA, 59 bp, synthetic construct
  source 1..59: mol_type = other DNA
tccctacacgacgctcttccgatctacaacacaacacagctcaggtatgcacgtcacga

SEQ ID NO: 255 - DNA, 59 bp, synthetic construct
  source 1..59: mol_type = other DNA
tccctacacgacgctcttccgatctacaacagatcacagctcaggtatgcacgtcacga

SEQ ID NO: 256 - DNA, 59 bp, synthetic construct
  source 1..59: mol_type = other DNA
tccctacacgacgctcttccgatctacaacagggcacagctcaggtatgcacgtcacga

SEQ ID NO: 257 - DNA, 59 bp, synthetic construct
  source 1..59: mol_type = other DNA
tccctacacgacgctcttccgatctacaacagtgcacagctcaggtatgcacgtcacga

SEQ ID NO: 258 - DNA, 59 bp, synthetic construct
  source 1..59: mol_type = other DNA
tccctacacgacgctcttccgatctaccacaacacacagctcaggtatgcacgtcacga

SEQ ID NO: 259 - DNA, 59 bp, synthetic construct
  source 1..59: mol_type = other DNA
tccctacacgacgctcttccgatctaccacattccacagctcaggtatgcacgtcacga

SEQ ID NO: 260 - DNA, 59 bp, synthetic construct
  source 1..59: mol_type = other DNA
tccctacacgacgctcttccgatctacgacaaagcacagctcaggtatgcacgtcacga

SEQ ID NO: 261 - DNA, 59 bp, synthetic construct
  source 1..59: mol_type = other DNA
tccctacacgacgctcttccgatctacgacatatcacagctcaggtatgcacgtcacga

SEQ ID NO: 262 - DNA, 59 bp, synthetic construct
  source 1..59: mol_type = other DNA
tccctacacgacgctcttccgatctactacacgccacagctcaggtatgcacgtcacga

SEQ ID NO: 263 - DNA, 59 bp, synthetic construct
  source 1..59: mol_type = other DNA
tccctacacgacgctcttccgatctactacagatcacagctcaggtatgcacgtcacga

SEQ ID NO: 264 - RNA, 59 nt, synthetic construct
  source 1..59: mol_type = other RNA
tccctacacgacgctcttccgatctactacatgacacagctcaggtatgcacgtcacga

SEQ ID NO: 265 - DNA, 59 bp, synthetic construct
  source 1..59: mol_type = other DNA
tccctacacgacgctcttccgatctagtacacaacacagctcaggtatgcacgtcacga

SEQ ID NO: 266 - DNA, 59 bp, synthetic construct
  source 1..59: mol_type = other DNA
tccctacacgacgctcttccgatctagtacacgtcacagctcaggtatgcacgtcacga

SEQ ID NO: 267 - DNA, 59 bp, synthetic construct
  source 1..59: mol_type = other DNA
tccctacacgacgctcttccgatctagtacatcccacagctcaggtatgcacgtcacga

SEQ ID NO: 268 - DNA, 59 bp, synthetic construct
  source 1..59: mol_type = other DNA
tccctacacgacgctcttccgatctataacacgtcacagctcaggtatgcacgtcacga

SEQ ID NO: 269 - DNA, 59 bp, synthetic construct
  source 1..59: mol_type = other DNA
tccctacacgacgctcttccgatctatcacaacgcacagctcaggtatgcacgtcacga

SEQ ID NO: 270 - DNA, 59 bp, synthetic construct
  source 1..59: mol_type = other DNA
tccctacacgacgctcttccgatctatgacaagccacagctcaggtatgcacgtcacga

SEQ ID NO: 271 - DNA, 59 bp, synthetic construct
  source 1..59: mol_type = other DNA
tccctacacgacgctcttccgatctatgacatcacacagctcaggtatgcacgtcacga

SEQ ID NO: 272 - DNA, 59 bp, synthetic construct
  source 1..59: mol_type = other DNA
tccctacacgacgctcttccgatctattacacctcacagctcaggtatgcacgtcacga

SEQ ID NO: 273 - DNA, 59 bp, synthetic construct
  source 1..59: mol_type = other DNA
tccctacacgacgctcttccgatctcaaacactacacagctcaggtatgcacgtcacga

SEQ ID NO: 274 - DNA, 59 bp, synthetic construct
  source 1..59: mol_type = other DNA
tccctacacgacgctcttccgatctcaatctaagcacagctcaggtatgcacgtcacga

SEQ ID NO: 275 - DNA, 59 bp, synthetic construct
  source 1..59: mol_type = other DNA
tccctacacgacgctcttccgatctcacacaagtcacagctcaggtatgcacgtcacga

SEQ ID NO: 276 - DNA, 59 bp, synthetic construct
  source 1..59: mol_type = other DNA
tccctacacgacgctcttccgatctcacacacggcacagctcaggtatgcacgtcacga

SEQ ID NO: 277 - DNA, 59 bp, synthetic construct
  source 1..59: mol_type = other DNA
tccctacacgacgctcttccgatctcacacagatcacagctcaggtatgcacgtcacga

SEQ ID NO: 278 - DNA, 59 bp, synthetic construct
  source 1..59: mol_type = other DNA
tccctacacgacgctcttccgatctcacacatcacacagctcaggtatgcacgtcacga

SEQ ID NO: 279 - DNA, 59 bp, synthetic construct
  source 1..59: mol_type = other DNA
tccctacacgacgctcttccgatctcagacaatccacagctcaggtatgcacgtcacga

SEQ ID NO: 280 - DNA, 59 bp, synthetic construct
  source 1..59: mol_type = other DNA
tccctacacgacgctcttccgatctcagacagcgcacagctcaggtatgcacgtcacga

SEQ ID NO: 281 - DNA, 59 bp, synthetic construct
  source 1..59: mol_type = other DNA
tccctacacgacgctcttccgatctcagacatcacacagctcaggtatgcacgtcacga

SEQ ID NO: 282 - DNA, 59 bp, synthetic construct
  source 1..59: mol_type = other DNA
tccctacacgacgctcttccgatctcatacacgacacagctcaggtatgcacgtcacga

SEQ ID NO: 283 - DNA, 59 bp, synthetic construct
  source 1..59: mol_type = other DNA
tccctacacgacgctcttccgatctcatacaggccacagctcaggtatgcacgtcacga

SEQ ID NO: 284 - DNA, 59 bp, synthetic construct
  source 1..59: mol_type = other DNA
tccctacacgacgctcttccgatctcatacatttcacagctcaggtatgcacgtcacga

SEQ ID NO: 285 - DNA, 59 bp, synthetic construct
  source 1..59: mol_type = other DNA
tccctacacgacgctcttccgatctccaacaacacacagctcaggtatgcacgtcacga

SEQ ID NO: 286 - DNA, 59 bp, synthetic construct
  source 1..59: mol_type = other DNA
tccctacacgacgctcttccgatctccgacaaaacacagctcaggtatgcacgtcacga

SEQ ID NO: 287 - DNA, 59 bp, synthetic construct
  source 1..59: mol_type = other DNA
tccctacacgacgctcttccgatctccgacatcccacagctcaggtatgcacgtcacga

SEQ ID NO: 288 - DNA, 59 bp, synthetic construct
  source 1..59: mol_type = other DNA
tccctacacgacgctcttccgatctcctacataacacagctcaggtatgcacgtcacga

SEQ ID NO: 289 - DNA, 59 bp, synthetic construct
  source 1..59: mol_type = other DNA
tccctacacgacgctcttccgatctcctacatggcacagctcaggtatgcacgtcacga

SEQ ID NO: 290 - DNA, 59 bp, synthetic construct
  source 1..59: mol_type = other DNA
tccctacacgacgctcttccgatctcgaacatgtcacagctcaggtatgcacgtcacga

SEQ ID NO: 291 - DNA, 59 bp, synthetic construct
  source 1..59: mol_type = other DNA
tccctacacgacgctcttccgatctcgcacaacgcacagctcaggtatgcacgtcacga

SEQ ID NO: 292 - DNA, 59 bp, synthetic construct
  source 1..59: mol_type = other DNA
tccctacacgacgctcttccgatctcggacaaatcacagctcaggtatgcacgtcacga

SEQ ID NO: 293 - DNA, 59 bp, synthetic construct
  source 1..59: mol_type = other DNA
tccctacacgacgctcttccgatctcggacatttcacagctcaggtatgcacgtcacga

SEQ ID NO: 294 - DNA, 59 bp, synthetic construct
  source 1..59: mol_type = other DNA
tccctacacgacgctcttccgatctcgtacaacgcacagctcaggtatgcacgtcacga

SEQ ID NO: 295 - DNA, 59 bp, synthetic construct
  source 1..59: mol_type = other DNA
tccctacacgacgctcttccgatctcgtacactacacagctcaggtatgcacgtcacga

SEQ ID NO: 296 - DNA, 59 bp, synthetic construct
  source 1..59: mol_type = other DNA
tccctacacgacgctcttccgatctcgtacatagcacagctcaggtatgcacgtcacga

SEQ ID NO: 297 - DNA, 59 bp, synthetic construct
  source 1..59: mol_type = other DNA
tccctacacgacgctcttccgatctctaacaccgcacagctcaggtatgcacgtcacga

SEQ ID NO: 298 - DNA, 59 bp, synthetic construct
  source 1..59: mol_type = other DNA
tccctacacgacgctcttccgatctctaacagctcacagctcaggtatgcacgtcacga

SEQ ID NO: 299 - DNA, 59 bp, synthetic construct
  source 1..59: mol_type = other DNA
tccctacacgacgctcttccgatctctaacataccacagctcaggtatgcacgtcacga

SEQ ID NO: 300 - DNA, 59 bp, synthetic construct
  source 1..59: mol_type = other DNA
tccctacacgacgctcttccgatctctcacaagacacagctcaggtatgcacgtcacga

SEQ ID NO: 301 - DNA, 59 bp, synthetic construct
  source 1..59: mol_type = other DNA
tccctacacgacgctcttccgatctcttacaacccacagctcaggtatgcacgtcacga

SEQ ID NO: 302 - DNA, 59 bp, synthetic construct
  source 1..59: mol_type = other DNA
tccctacacgacgctcttccgatctcttacagtacacagctcaggtatgcacgtcacga

SEQ ID NO: 303 - DNA, 59 bp, synthetic construct
  source 1..59: mol_type = other DNA
tccctacacgacgctcttccgatctgaaacagctcacagctcaggtatgcacgtcacga

SEQ ID NO: 304 - DNA, 59 bp, synthetic construct
  source 1..59: mol_type = other DNA
tccctacacgacgctcttccgatctgaaacatcgcacagctcaggtatgcacgtcacga

SEQ ID NO: 305 - DNA, 59 bp, synthetic construct
  source 1..59: mol_type = other DNA
tccctacacgacgctcttccgatctgacacatgacacagctcaggtatgcacgtcacga

SEQ ID NO: 306 - DNA, 59 bp, synthetic construct
  source 1..59: mol_type = other DNA
tccctacacgacgctcttccgatctgagacaactcacagctcaggtatgcacgtcacga

SEQ ID NO: 307 - DNA, 59 bp, synthetic construct
  source 1..59: mol_type = other DNA
tccctacacgacgctcttccgatctgagacactacacagctcaggtatgcacgtcacga

SEQ ID NO: 308 - DNA, 59 bp, synthetic construct
  source 1..59: mol_type = other DNA
tccctacacgacgctcttccgatctgagacatggcacagctcaggtatgcacgtcacga

SEQ ID NO: 309 - DNA, 59 bp, synthetic construct
  source 1..59: mol_type = other DNA
tccctacacgacgctcttccgatctgatacacagcacagctcaggtatgcacgtcacga

SEQ ID NO: 310 - DNA, 59 bp, synthetic construct
  source 1..59: mol_type = other DNA
tccctacacgacgctcttccgatctgatacagatcacagctcaggtatgcacgtcacga

SEQ ID NO: 311 - DNA, 59 bp, synthetic construct
  source 1..59: mol_type = other DNA
tccctacacgacgctcttccgatctgccacaaatcacagctcaggtatgcacgtcacga

SEQ ID NO: 312 - DNA, 59 bp, synthetic construct
  source 1..59: mol_type = other DNA
tccctacacgacgctcttccgatctgcgacactacacagctcaggtatgcacgtcacga

SEQ ID NO: 313 - DNA, 59 bp, synthetic construct
  source 1..59: mol_type = other DNA
tccctacacgacgctcttccgatctggaacacaccacagctcaggtatgcacgtcacga

SEQ ID NO: 314 - DNA, 59 bp, synthetic construct
  source 1..59: mol_type = other DNA
tccctacacgacgctcttccgatctggcacataccacagctcaggtatgcacgtcacga

SEQ ID NO: 315 - DNA, 59 bp, synthetic construct
  source 1..59: mol_type = other DNA
tccctacacgacgctcttccgatctggtacaagccacagctcaggtatgcacgtcacga

SEQ ID NO: 316 - DNA, 59 bp, synthetic construct
  source 1..59: mol_type = other DNA
tccctacacgacgctcttccgatctgtaacagagcacagctcaggtatgcacgtcacga

SEQ ID NO: 317 - DNA, 59 bp, synthetic construct
  source 1..59: mol_type = other DNA
tccctacacgacgctcttccgatctgtaacagtccacagctcaggtatgcacgtcacga

SEQ ID NO: 318 - DNA, 59 bp, synthetic construct
  source 1..59: mol_type = other DNA
tccctacacgacgctcttccgatctgtcacacgccacagctcaggtatgcacgtcacga

SEQ ID NO: 319 - DNA, 59 bp, synthetic construct
  source 1..59: mol_type = other DNA
tccctacacgacgctcttccgatctgtgacaaaacacagctcaggtatgcacgtcacga

SEQ ID NO: 320 - DNA, 59 bp, synthetic construct
  source 1..59: mol_type = other DNA
tccctacacgacgctcttccgatctgtgacagcccacagctcaggtatgcacgtcacga

SEQ ID NO: 321 - DNA, 59 bp, synthetic construct
  source 1..59: mol_type = other DNA
tccctacacgacgctcttccgatctgttacaacgcacagctcaggtatgcacgtcacga

SEQ ID NO: 322 - DNA, 59 bp, synthetic construct
  source 1..59: mol_type = other DNA
tccctacacgacgctcttccgatctgttacatcacacagctcaggtatgcacgtcacga

SEQ ID NO: 323 - DNA, 59 bp, synthetic construct
  source 1..59: mol_type = other DNA
tccctacacgacgctcttccgatcttaaacaggccacagctcaggtatgcacgtcacga

SEQ ID NO: 324 - DNA, 59 bp, synthetic construct
  source 1..59: mol_type = other DNA
tccctacacgacgctcttccgatcttaaacatcgcacagctcaggtatgcacgtcacga

SEQ ID NO: 325 - DNA, 59 bp, synthetic construct
  source 1..59: mol_type = other DNA
tccctacacgacgctcttccgatcttaaacatgtcacagctcaggtatgcacgtcacga

SEQ ID NO: 326 - DNA, 59 bp, synthetic construct
  source 1..59: mol_type = other DNA
tccctacacgacgctcttccgatcttacacaagccacagctcaggtatgcacgtcacga

SEQ ID NO: 327 - DNA, 59 bp, synthetic construct
  source 1..59: mol_type = other DNA
tccctacacgacgctcttccgatcttacacaatacacagctcaggtatgcacgtcacga

SEQ ID NO: 328 - DNA, 59 bp, synthetic construct
  source 1..59: mol_type = other DNA
tccctacacgacgctcttccgatcttacacaatccacagctcaggtatgcacgtcacga

SEQ ID NO: 329 - DNA, 59 bp, synthetic construct
  source 1..59: mol_type = other DNA
tccctacacgacgctcttccgatcttacacacagcacagctcaggtatgcacgtcacga

SEQ ID NO: 330 - DNA, 59 bp, synthetic construct
  source 1..59: mol_type = other DNA
tccctacacgacgctcttccgatcttagacacttcacagctcaggtatgcacgtcacga

SEQ ID NO: 331 - DNA, 59 bp, synthetic construct
  source 1..59: mol_type = other DNA
tccctacacgacgctcttccgatcttatacaaatcacagctcaggtatgcacgtcacga

SEQ ID NO: 332 - DNA, 59 bp, synthetic construct
  source 1..59: mol_type = other DNA
tccctacacgacgctcttccgatcttatacacagcacagctcaggtatgcacgtcacga

SEQ ID NO: 333 - DNA, 59 bp, synthetic construct
  source 1..59: mol_type = other DNA
tccctacacgacgctcttccgatcttcaacatgacacagctcaggtatgcacgtcacga

SEQ ID NO: 334 - DNA, 59 bp, synthetic construct
  source 1..59: mol_type = other DNA
tccctacacgacgctcttccgatcttcaacatgtcacagctcaggtatgcacgtcacga

SEQ ID NO: 335 - DNA, 59 bp, synthetic construct
  source 1..59: mol_type = other DNA
tccctacacgacgctcttccgatcttcaacattccacagctcaggtatgcacgtcacga

SEQ ID NO: 336 - DNA, 59 bp, synthetic construct
  source 1..59: mol_type = other DNA
tccctacacgacgctcttccgatcttccacacagcacagctcaggtatgcacgtcacga

SEQ ID NO: 337 - DNA, 59 bp, synthetic construct
  source 1..59: mol_type = other DNA
tccctacacgacgctcttccgatcttccacactacacagctcaggtatgcacgtcacga

SEQ ID NO: 338 - DNA, 59 bp, synthetic construct
  source 1..59: mol_type = other DNA
tccctacacgacgctcttccgatcttcgacaaagcacagctcaggtatgcacgtcacga

SEQ ID NO: 339 - DNA, 59 bp, synthetic construct
  source 1..59: mol_type = other DNA
tccctacacgacgctcttccgatcttcgacaacacacagctcaggtatgcacgtcacga

SEQ ID NO: 340 - DNA, 59 bp, synthetic construct
  source 1..59: mol_type = other DNA
tccctacacgacgctcttccgatcttcgacactccacagctcaggtatgcacgtcacga

SEQ ID NO: 341 - DNA, 59 bp, synthetic construct
  source 1..59: mol_type = other DNA
tccctacacgacgctcttccgatcttcgacagcacacagctcaggtatgcacgtcacga

SEQ ID NO: 342 - DNA, 59 bp, synthetic construct
  source 1..59: mol_type = other DNA
tccctacacgacgctcttccgatcttgaacaccacacagctcaggtatgcacgtcacga

SEQ ID NO: 343 - DNA, 59 bp, synthetic construct
  source 1..59: mol_type = other DNA
tccctacacgacgctcttccgatcttgaacatgacacagctcaggtatgcacgtcacga

SEQ ID NO: 344 - DNA, 59 bp, synthetic construct
  source 1..59: mol_type = other DNA
tccctacacgacgctcttccgatcttgtacatcacacagctcaggtatgcacgtcacga

SEQ ID NO: 345 - DNA, 59 bp, synthetic construct
  source 1..59: mol_type = other DNA
tccctacacgacgctcttccgatctttaacaggccacagctcaggtatgcacgtcacga

SEQ ID NO: 346 - DNA, 59 bp, synthetic construct
  source 1..59: mol_type = other DNA
tccctacacgacgctcttccgatctttcacacggcacagctcaggtatgcacgtcacga

SEQ ID NO: 347 - DNA, 59 bp, synthetic construct
  source 1..59: mol_type = other DNA
tccctacacgacgctcttccgatctttgacatcgcacagctcaggtatgcacgtcacga

SEQ ID NO: 348 - DNA, 59 bp, synthetic construct
  source 1..59: mol_type = other DNA
tccctacacgacgctcttccgatcttttacaccgcacagctcaggtatgcacgtcacga

SEQ ID NO: 349 - DNA, 59 bp, synthetic construct
  source 1..59: mol_type = other DNA
tccctacacgacgctcttccgatcttttacagagcacagctcaggtatgcacgtcacga

SEQ ID NO: 350 - DNA, 64 bp, synthetic construct
  source 1..64: mol_type = other DNA
caagcagaagacggcatacgagatcgtgatgtgactggagttcagacgtgtgctcttccgatct

SEQ ID NO: 351 - DNA, 64 bp, synthetic construct
  source 1..64: mol_type = other DNA
caagcagaagacggcatacgagatacatcggtgactggagttcagacgtgtgctcttccgatct

SEQ ID NO: 352 - DNA, 64 bp, synthetic construct
  source 1..64: mol_type = other DNA
caagcagaagacggcatacgagatgcctaagtgactggagttcagacgtgtgctcttccgatct

SEQ ID NO: 353 - DNA, 64 bp, synthetic construct
  source 1..64: mol_type = other DNA
caagcagaagacggcatacgagattggtctgtgactggagttcagacgtgtgctcttccgatct

SEQ ID NO: 354 - DNA, 64 bp, synthetic construct
  source 1..64: mol_type = other DNA
caagcagaagacggcatacgagatcactgtgtgactggagttcagacgtgtgctcttccgatct

SEQ ID NO: 355 - DNA, 64 bp, synthetic construct
  source 1..64: mol_type = other DNA
caagcagaagacggcatacgagatattggcgtgactggagttcagacgtgtgctcttccgatct

SEQ ID NO: 356 - DNA, 64 bp, synthetic construct
  source 1..64: mol_type = other DNA
caagcagaagacggcatacgagatgatctggtgactggagttcagacgtgtgctcttccgatct

SEQ ID NO: 357 - DNA, 64 bp, synthetic construct
  source 1..64: mol_type = other DNA
caagcagaagacggcatacgagattcaagtgtgactggagttcagacgtgtgctcttccgatct

SEQ ID NO: 358 - DNA, 64 bp, synthetic construct
  source 1..64: mol_type = other DNA
caagcagaagacggcatacgagatctgatcgtgactggagttcagacgtgtgctcttccgatct

SEQ ID NO: 359 - DNA, 64 bp, synthetic construct
  source 1..64: mol_type = other DNA
caagcagaagacggcatacgagataagctagtgactggagttcagacgtgtgctcttccgatct

SEQ ID NO: 360 - DNA, 64 bp, synthetic construct
  source 1..64: mol_type = other DNA
caagcagaagacggcatacgagatgtagccgtgactggagttcagacgtgtgctcttccgatct

SEQ ID NO: 361 - DNA, 64 bp, synthetic construct
  source 1..64: mol_type = other DNA
caagcagaagacggcatacgagattacaaggtgactggagttcagacgtgtgctcttccgatct

SEQ ID NO: 362 - DNA, 64 bp, synthetic construct
  source 1..64: mol_type = other DNA
caagcagaagacggcatacgagatttgactgtgactggagttcagacgtgtgctcttccgatct

SEQ ID NO: 363 - DNA, 64 bp, synthetic construct
  source 1..64: mol_type = other DNA
caagcagaagacggcatacgagatggaactgtgactggagttcagacgtgtgctcttccgatct

SEQ ID NO: 364 - DNA, 64 bp, synthetic construct
  source 1..64: mol_type = other DNA
caagcagaagacggcatacgagattgacatgtgactggagttcagacgtgtgctcttccgatct

SEQ ID NO: 365 - DNA, 64 bp, synthetic construct
  source 1..64: mol_type = other DNA
caagcagaagacggcatacgagatggacgggtgactggagttcagacgtgtgctcttccgatct

SEQ ID NO: 366 - DNA, 64 bp, synthetic construct
  source 1..64: mol_type = other DNA
caagcagaagacggcatacgagatgcggacgtgactggagttcagacgtgtgctcttccgatct

SEQ ID NO: 367 - DNA, 64 bp, synthetic construct
  source 1..64: mol_type = other DNA
caagcagaagacggcatacgagattttcacgtgactggagttcagacgtgtgctcttccgatct

SEQ ID NO: 368 - DNA, 64 bp, synthetic construct
  source 1..64: mol_type = other DNA
caagcagaagacggcatacgagatggccacgtgactggagttcagacgtgtgctcttccgatct

SEQ ID NO: 369 - DNA, 64 bp, synthetic construct
  source 1..64: mol_type = other DNA
caagcagaagacggcatacgagatcgaaacgtgactggagttcagacgtgtgctcttccgatct

SEQ ID NO: 370 - DNA, 64 bp, synthetic construct
  source 1..64: mol_type = other DNA
caagcagaagacggcatacgagatcgtacggtgactggagttcagacgtgtgctcttccgatct

SEQ ID NO: 371 - DNA, 64 bp, synthetic construct
  source 1..64: mol_type = other DNA
caagcagaagacggcatacgagatccactcgtgactggagttcagacgtgtgctcttccgatct

SEQ ID NO: 372 - DNA, 64 bp, synthetic construct
  source 1..64: mol_type = other DNA
caagcagaagacggcatacgagatatcagtgtgactggagttcagacgtgtgctcttccgatct

SEQ ID NO: 373 - DNA, 64 bp, synthetic construct
  source 1..64: mol_type = other DNA
caagcagaagacggcatacgagataggaatgtgactggagttcagacgtgtgctcttccgatct

SEQ ID NO: 374 - DNA, 44 bp, synthetic construct
  source 1..44: mol_type = other DNA
aatgatacggcgaccaccgagatctacactctttccctacacga

SEQ ID NO: 375 - DNA, 56 bp, synthetic construct
  source 1..56: mol_type = other DNA
gtagcacccactgcactgacgthhhachhhcctcaaccctgcacgcacacactctg

SEQ ID NO: 376 - DNA, 54 bp, synthetic construct
  source 1..54: mol_type = other DNA
gtagcacccactgcactgacgthhhachhhcgaggggtaactcatgagcagtgg

SEQ ID NO: 377 - DNA, 60 bp, synthetic construct
  source 1..60: mol_type = other DNA
gtagcacccactgcactgacgthhhachhhcaggccaaagaattcctggaaggtgttcag

SEQ ID NO: 378 - DNA, 55 bp, synthetic construct
  source 1..55: mol_type = other DNA
gtagcacccactgcactgacgthhhachhhttatggcagtggcagctctctgagc

SEQ ID NO: 379 - DNA, 51 bp, synthetic construct
  source 1..51: mol_type = other DNA
cacagctcaggtatgcacgtcacgagcctggagtttctcaggccctgctcc

SEQ ID NO: 380 - DNA, 44 bp, synthetic construct
  source 1..44: mol_type = other DNA
cacagctcaggtatgcacgtcacgaccatccccacctccacagc

SEQ ID NO: 381 - DNA, 51 bp, synthetic construct
  source 1..51: mol_type = other DNA
cacagctcaggtatgcacgtcacgagggacggtcacctttggggtggtgac

SEQ ID NO: 382 - DNA, 51 bp, synthetic construct
  source 1..51: mol_type = other DNA
cacagctcaggtatgcacgtcacgaggctgcttagctggcttgccgcttcc

SEQ ID NO: 383 - skipped